European Patent Application EP 4 253 421 A2, published October 4, 2023. Title: Anti-HER2 Biparatopic Antibody-Drug Conjugates and Methods of Use. Applicant: ZYMEWORKS BC INC. The sequence listing filed with the application follows.

SEQUENCE LISTING (89 sequences)

SEQ ID NO: 1 - protein, 217 aa, synthetic construct
  REGION 1..217: note = Artificial sequence
APELLGGPSVFLFPPKPKDTLMISRTPEVTCVVVDVSHEDPEVKFNWYVDGVEVHNAKTKPREEQYNSTYRVVSVLTVLHQDWLNGKEYKCKVSNKALPAPIEKTISKAKGQPREPQVYTLPPSRDELTKNQVSLTCLVKGFYPSDIAVEWESNGQPENNYKTTPPVLDSDGSFFLYSKLTVDKSRWQQGNVFSCSVMHEALHNHYTQKSLSLSPGK

SEQ ID NO: 2 - protein, 607 aa, Homo sapiens
TQVCTGTDMKLRLPASPETHLDMLRHLYQGCQVVQGNLELTYLPTNASLSFLQDIQEVQGYVLIAHNQVRQVPLQRLRIVRGTQLFEDNYALAVLDNGDPLNNTTPVTGASPGGLRELQLRSLTEILKGGVLIQRNPQLCYQDTILWKDIFHKNNQLALTLIDTNRSRACHPCSPMCKGSRCWGESSEDCQSLTRTVCAGGCARCKGPLPTDCCHEQCAAGCTGPKHSDCLACLHFNHSGICELHCPALVTYNTDTFESMPNPEGRYTFGASCVTACPYNYLSTDVGSCTLVCPLHNQEVTAEDGTQRCEKCSKPCARVCYGLGMEHLREVRAVTSANIQEFAGCKKIFGSLAFLPESFDGDPASNTAPLQPEQLQVFETLEEITGYLYISAWPDSLPDLSVFQNLQVIRGRILHNGAYSLTLQGLGISWLGLRSLRELGSGLALIHHNTHLCFVHTVPWDQLFRNPHQALLHTANRPEDECVGEGLACHQLCARGHCWGPGPTQCVNCSQFLRGQECVEECRVLQGLPREYVNARHCLPCHPECQPQNGSVTCFGPEADQCVACAHYKDPPFCVARCPSGVKPDLSYMPIWKFPDEEGACQPCPIN

SEQ ID NO: 3 - protein, 448 aa, synthetic construct
  REGION 1..448: note = Artificial sequence
EVQLVESGGGLVQPGGSLRLSCAASGFTFTDYTMDWVRQAPGKGLEWVADVNPNSGGSIYNQRFKGRFTLSVDRSKNTLYLQMNSLRAEDTAVYYCARNLGPSFYFDYWGQGTLVTVSSASTKGPSVFPLAPSSKSTSGGTAALGCLVKGYFPEPVTVSWNSGALTSGVHTFPAVLKSSGLYSLSSVVTVPSSSLGTQTYICNVNHKPSNTKVDKKVEPKSCDKTHTCPPCPAPELLGGPSVFLFPPKPKDTLMISRTPEVTCVVVDVSHEDPEVKFNWYVDGVEVHNAKTKPREEQYNSTYRVVSVLTVLHQDWLNGKEYKCKVSNKALPAPIEKTISKAKGQPREPQVYVLPPSRDELTKNQVSLLCLVKGFYPSDIAVEWESNGQPENNYLTWPPVLDSDGSFFLYSKLTVDKSRWQQGNVFSCSVMHEALHNHYTQKSLSLSPG

SEQ ID NO: 4 - DNA, 1344 bp, synthetic construct
  misc_feature 1..1344: note = Artificial Sequence
  source 1..1344: mol_type = other DNA
gaagtgcagctggtcgaatctggaggaggactggtgcagccaggagggtccctgcgcctgtcttgcgccgctagtggcttcacttttaccgactacaccatggattgggtgcgacaggcacctggaaagggcctggagtgggtcgccgatgtgaacccaaatagcggaggctccatctacaaccagcggttcaagggccggttcaccctgtcagtggaccggagcaaaaacaccctgtatctgcagatgaatagcctgcgagccgaagatactgctgtgtactattgcgcccggaatctggggccctccttctactttgactattgggggcagggaactctggtcaccgtgagctccgcctccaccaagggaccttctgtgttcccactggctccctctagtaaatccacatctgggggaactgcagccctgggctgtctggtgaagggctacttcccagagcccgtcacagtgtcttggaacagtggcgctctgacttctggggtccacacctttcctgcagtgctgaagtcaagcgggctgtacagcctgtcctctgtggtcaccgtgccaagttcaagcctgggaacacagacttatatctgcaacgtgaatcacaagccatccaatacaaaagtcgacaagaaagtggaacccaagtcttgtgataaaacccatacatgccccccttgtcctgcaccagagctgctgggaggaccaagcgtgttcctgtttccacccaagcctaaagatacactgatgattagtaggaccccagaagtcacatgcgtggtcgtggacgtgagccacgaggaccccgaagtcaagtttaactggtacgtggacggcgtcgaggtgcataatgccaagactaaacccagggaggaacagtacaacagtacctatcgcgtcgtgtcagtcctgacagtgctgcatcaggattggctgaacgggaaagagtataagtgcaaagtgagcaataaggctctgcccgcacctatcgagaaaacaatttccaaggcaaaaggacagcctagagaaccacaggtgtacgtgctgcctccatcaagggatgagctgacaaagaaccaggtcagcctgctgtgtctggtgaaaggattctatccctctgacattgctgtggagtgggaaagtaatggccagcctgagaacaattacctgacctggccccctgtgctggactcagatggcagcttctttctgtatagcaagctgaccgtcgacaaatcccggtggcagcaggggaatgtgtttagttgttcagtcatgcacgaggcactgcacaaccattacacccagaagtcactgtcactgtcaccaggg

SEQ ID NO: 5 - protein, 119 aa, synthetic construct [sequence omitted]

SEQ ID NO: 6 - protein, 8 aa, synthetic construct
  REGION 1..8: note = Artificial sequence
GFTFTDYT

SEQ ID NO: 7 - protein, 12 aa, synthetic construct
  REGION 1..12: note = Artificial sequence
ARNLGPSFYFDY

SEQ ID NO: 8 - protein, 8 aa, synthetic construct
  REGION 1..8: note = Artificial sequence
VNPNSGGS

SEQ ID NO: 9 - protein, 214 aa, synthetic construct
  REGION 1..214: note = Artificial sequence
DIQMTQSPSSLSASVGDRVTITCKASQDVSIGVAWYQQKPGKAPKLLIYSASYRYTGVPSRFSGSGSGTDFTLTISSLQPEDFATYYCQQYYIYPYTFGQGTKVEIKRTVAAPSVFIFPPSDEQLKSGTASVVCLLNNFYPREAKVQWKVDNALQSGNSQESVTEQDSKDSTYSLSSTLTLSKADYEKHKVYACEVTHQGLSSPVTKSFNRGEC

SEQ ID NO: 10 - DNA, 642 bp, synthetic construct
  misc_feature 1..642: note = Artificial sequence
  source 1..642: mol_type = other DNA
gatattcagatgacccagtccccaagctccctgagtgcctcagtgggcgaccgagtcaccatcacatgcaaggcttcccaggatgtgtctattggagtcgcatggtaccagcagaagccaggcaaagcacccaagctgctgatctatagcgcctcctaccggtataccggcgtgccctctagattctctggcagtgggtcaggaacagactttactctgaccatctctagtctgcagcctgaggatttcgctacctactattgccagcagtactatatctacccatatacctttggccaggggacaaaagtggagatcaagaggactgtggccgctccctccgtcttcatttttcccccttctgacgaacagctgaaaagtggcacagccagcgtggtctgtctgctgaacaatttctaccctcgcgaagccaaagtgcagtggaaggtcgataacgctctgcagagcggcaacagccaggagtctgtgactgaacaggacagtaaagattcaacctatagcctgtcaagcacactgactctgagcaaggcagactacgagaagcacaaagtgtatgcctgcgaagtcacacatcaggggctgtcctctcctgtgactaagagctttaacagaggagagtgt

SEQ ID NO: 11 - protein, 107 aa, synthetic construct [sequence omitted]

SEQ ID NO: 12 - protein, 6 aa, synthetic construct
  REGION 1..6: note = Artificial sequence
QDVSIG

SEQ ID NO: 13 - protein, 9 aa, synthetic construct
  REGION 1..9: note = Artificial sequence
QQYYIYPYT

SEQ ID NO: 14 - skipped

SEQ ID NO: 15 - protein, 222 aa, synthetic construct
  REGION 1..222: note = Artificial sequence
DYKDDDDKDIQMTQSPSSLSASVGDRVTITCRASQDVNTAVAWYQQKPGKAPKLLIYSASFLYSGVPSRFSGSRSGTDFTLTISSLQPEDFATYYCQQHYTTPPTFGQGTKVEIKRTVAAPSVFIFPPSDERLKSGTASVVCLLNNFYPREAKVQWKVDNALQSGNSQESVTEQDSKDSTYSLSSTLTLSKADYEKHKVYACEVTHQGLSSPVTKSFNRGEC

SEQ ID NO: 16 - DNA, 666 bp, synthetic construct
  misc_feature 1..666: note = Artificial sequence
  source 1..666: mol_type = other DNA
gactacaaagacgacgatgacaaagatatccagatgacccagtcccctagctccctgtccgcttctgtgggcgatagggtcactattacctgccgcgcatctcaggacgtgaacaccgcagtcgcctggtaccagcagaagcctgggaaagctccaaagctgctgatctacagtgcatcattcctgtattcaggagtgcccagccggtttagcggcagcagatctggcaccgatttcacactgactatttctagtctgcagcctgaggactttgccacatactattgccagcagcactataccacaccccctactttcggccaggggaccaaagtggagatcaagcgaactgtggccgctccaagtgtcttcatttttccacccagcgatgaaagactgaagtccggcacagcttctgtggtctgtctgctgaacaatttttaccccagagaggccaaagtgcagtggaaggtcgacaacgctctgcagagtggcaacagccaggagagcgtgacagaacaggattccaaagactctacttatagtctgtcaagcaccctgacactgagcaaggcagactacgaaaagcataaagtgtatgcctgtgaggtcacacatcaggggctgtcatcaccagtcaccaaatcattcaatcggggggagtgc

SEQ ID NO: 17 - protein, 107 aa, synthetic construct [sequence omitted]

SEQ ID NO: 18 - protein, 222 aa, synthetic construct
  REGION 1..222: note = Artificial sequence
DYKDDDDKDIQMTQSPSSLSASVGDRVTITCRASQDVNTAVAWYQQKPGKAPKLLIYSASFLYSGVPSRFSGSRSGTDFTLTISSLQPEDFATYYCQQHYTTPPTFGQGTKVEIKRTVAAPSVFIFPPSDERLKSGTASVVCLLNNFYPREAKVQWKVDNALQSGNSKESVTEQDSKDSTYSLSSRLTLSKADYEKHKVYACEVTHQGLSSPVTKSFNRGEC

SEQ ID NO: 19 - DNA, 666 bp, synthetic construct
  misc_feature 1..666: note = Artificial sequence
  source 1..666: mol_type = other DNA
gactacaaagacgacgatgacaaagatatccagatgacccagtcccctagctccctgtccgcttctgtgggcgatagggtcactattacctgccgcgcatctcaggacgtgaacaccgcagtcgcctggtaccagcagaagcctgggaaagctccaaagctgctgatctacagtgcatcattcctgtattcaggagtgcccagccggtttagcggcagcagatctggcaccgatttcacactgactatttctagtctgcagcctgaggactttgccacatactattgccagcagcactataccacaccccctactttcggccaggggaccaaagtggagatcaagcgaactgtggccgctccaagtgtcttcatttttccacccagcgatgaaagactgaagtccggcacagcttctgtggtctgtctgctgaacaatttttaccccagagaggccaaagtgcagtggaaggtcgacaacgctctgcagagtggcaacagcaaggagagcgtgacagaacaggattccaaagactctacttatagtctgtcaagcagactgacactgagcaaggcagactacgaaaagcataaagtgtatgcctgtgaggtcacacatcaggggctgtcatcaccagtcaccaaatcattcaatcggggggagtgc

SEQ ID NO: 20 - protein, 107 aa, synthetic construct [sequence omitted]

SEQ ID NO: 21 - protein, 6 aa, synthetic construct
  REGION 1..6: note = Artificial sequence
QDVNTA

SEQ ID NO: 22 - protein, 9 aa, synthetic construct
  REGION 1..9: note = Artificial sequence
QQHYTTPPT

SEQ ID NO: 23 - skipped

SEQ ID NO: 24 - protein, 214 aa, synthetic construct
  REGION 1..214: note = Artificial sequence
DIQMTQSPSSLSASVGDRVTITCKASQDVSIGVAWYQQKPGKAPKLLIYSASYRYTGVPSRFSGSGSGTDFTLTISSLQPEDFATYYCQQYYIYPATFGQGTKVEIKRTVAAPSVFIFPPSDEQLKSGTASVVCLLNNFYPREAKVQWKVDNALQSGNSQESVTEQDSKDSTYSLSSTLTLSKADYEKHKVYACEVTHQGLSSPVTKSFNRGEC

SEQ ID NO: 25 - DNA, 642 bp, synthetic construct
  misc_feature 1..642: note = Artificial sequence
  source 1..642: mol_type = other DNA
gatattcagatgacccagtccccaagctccctgagtgcctcagtgggcgaccgagtcaccatcacatgcaaggcttcccaggatgtgtctattggagtcgcatggtaccagcagaagccaggcaaagcacccaagctgctgatctatagcgcctcctaccggtataccggcgtgccctctagattctctggcagtgggtcaggaacagactttactctgaccatctctagtctgcagcctgaggatttcgctacctactattgccagcagtactatatctacccagccacctttggccaggggacaaaagtggagatcaagaggactgtggccgctccctccgtcttcatttttcccccttctgacgaacagctgaaaagtggcacagccagcgtggtctgtctgctgaacaatttctaccctcgcgaagccaaagtgcagtggaaggtcgataacgctctgcagagcggcaacagccaggagtctgtgactgaacaggacagtaaagattcaacctatagcctgtcaagcacactgactctgagcaaggcagactacgagaagcacaaagtgtatgcctgcgaagtcacacatcaggggctgtcctctcctgtgactaagagctttaacagaggagagtgt

SEQ ID NO: 26 - protein, 107 aa, synthetic construct
  REGION 1..107: note = Artificial sequence
DIQMTQSPSSLSASVGDRVTITCKASQDVSIGVAWYQQKPGKAPKLLIYSASYRYTGVPSRFSGSGSGTDFTLTISSLQPEDFATYYCQQYYIYPATFGQGTKVEIK

SEQ ID NO: 27 - protein, 6 aa, synthetic construct
  REGION 1..6: note = Artificial sequence
QDVSIG

SEQ ID NO: 28 - protein, 9 aa, synthetic construct
  REGION 1..9: note = Artificial sequence
QQYYIYPAT

SEQ ID NO: 29 - skipped

SEQ ID NO: 30 - protein, 449 aa, synthetic construct
  REGION 1..449: note = Artificial sequence
EVQLVESGGGLVQPGGSLRLSCAASGFNIKDTYIHWVRQAPGKGLEWVARIYPTNGYTRYADSVKGRFTISADTSKNTAYLQMNSLRAEDTAVYYCSRWGGDGFYAMDYWGQGTLVTVSSASTKGPSVFPLAPSSKSTSGGTAALGCEVTDYFPEPVTVSWNSGALTSGVHTFPAVLQSSGLYSLSSVVTVPSSSLGTQTYICNVNHKPSNTKVDKKVEPKSCDKTHTCPPCPAPELLGGPSVFLFPPKPKDTLMISRTPEVTCVVVDVSHEDPEVKFNWYVDGVEVHNAKTKPREEQYNSTYRVVSVLTVLHQDWLNGKEYKCKVSNKALPAPIEKTISKAKGQPREPQVYVYPPSRDELTKNQVSLTCLVKGFYPSDIAVEWESNGQPENNYKTTPPVLDSDGSFALVSKLTVDKSRWQQGNVFSCSVMHEALHNHYTQKSLSLSPG

SEQ ID NO: 31 - DNA, 1347 bp, synthetic construct
  misc_feature 1..1347: note = Artificial sequence
  source 1..1347: mol_type = other DNA
gaggtgcagctggtcgaaagcggaggaggactggtgcagccaggagggtcactgcgactgagctgcgcagcttccggcttcaacatcaaggacacctacattcactgggtccgccaggctcctggaaaaggcctggagtgggtggcacgaatctatccaactaatggatacacccggtatgccgactccgtgaagggccggttcaccatttctgcagatacaagtaaaaacactgcctacctgcagatgaacagcctgcgagccgaagatacagccgtgtactattgcagccgatggggaggcgacggcttctacgctatggattattgggggcagggaaccctggtcacagtgagctccgcatcaacaaaggggcctagcgtgtttccactggccccctctagtaaatccacctctgggggaacagcagccctgggatgtgaggtgaccgactacttcccagagcccgtcactgtgagctggaactccggcgccctgacatctggggtccatacttttcctgctgtgctgcagtcaagcggcctgtacagcctgtcctctgtggtcactgtgccaagttcaagcctggggactcagacctatatctgcaacgtgaatcacaagccatccaataccaaagtcgacaagaaagtggaacccaagtcttgtgataaaacacatacttgccccccttgtcctgcaccagagctgctgggaggaccaagcgtgttcctgtttccacccaagcctaaagacaccctgatgattagtaggactccagaagtcacctgcgtggtcgtggacgtgagccacgaggaccccgaagtcaagttcaactggtacgtggatggcgtcgaggtgcataatgccaagacaaaacccagggaggaacagtacaactccacttatcgcgtcgtgtctgtcctgaccgtgctgcaccaggactggctgaacggcaaggagtataagtgcaaagtgagcaataaggctctgcccgcacctatcgagaaaacaatttccaaggctaaagggcagcctagagaaccacaggtgtacgtgtaccctccatctagggacgagctgaccaagaaccaggtcagtctgacatgtctggtgaaagggttctatcccagcgatatcgcagtggagtgggaatccaatggacagcctgagaacaattacaagaccacaccccctgtgctggactctgatggaagtttcgccctggtgagtaagctgaccgtcgataaatcacggtggcagcagggcaacgtgttcagctgttcagtgatgcacgaagcactgcacaaccactacacccagaaaagcctgtccctgtcccccggc

SEQ ID NO: 32 - protein, 120 aa, synthetic construct [sequence omitted]

SEQ ID NO: 33 - protein, 8 aa, synthetic construct
  REGION 1..8: note = Artificial sequence
GFNIKDTY

SEQ ID NO: 34 - protein, 13 aa, synthetic construct
  REGION 1..13: note = Artificial sequence
SRWGGDGFYAMDY

SEQ ID NO: 35 - protein, 8 aa, synthetic construct
  REGION 1..8: note = Artificial sequence
IYPTNGYT

SEQ ID NO: 36 - protein, 448 aa, synthetic construct
  REGION 1..448: note = Artificial sequence
EVQLVESGGGLVQPGGSLRLSCAASGFTFADYTMDWVRQAPGKGLEWVGDVNPNSGGSIYNQRFKGRFTFSVDRSKNTLYLQMNSLRAEDTAVYYCARNLGPSFYFDYWGQGTLVTVSSASTKGPSVFPLAPSSKSTSGGTAALGCLVKDYFPEPVTVSWNSGALTSGVHTFPAVLQSSGLYSLSSVVTVPSSSLGTQTYICNVNHKPSNTKVDKKVEPKSCDKTHTCPPCPAPELLGGPSVFLFPPKPKDTLMISRTPEVTCVVVDVSHEDPEVKFNWYVDGVEVHNAKTKPREEQYNSTYRVVSVLTVLHQDWLNGKEYKCKVSNKALPAPIEKTISKAKGQPREPQVYVYPPSRDELTKNQVSLTCLVKGFYPSDIAVEWESNGQPENNYKTTPPVLDSDGSFALVSKLTVDKSRWQQGNVFSCSVMHEALHNHYTQKSLSLSPG

SEQ ID NO: 37 - DNA, 1344 bp, synthetic construct
  misc_feature 1..1344: note = Artificial sequence
  source 1..1344: mol_type = other DNA
gaggtgcagctggtggaatcaggagggggcctggtgcagcccggagggtctctgcgactgtcatgtgccgcttctgggttcactttcgcagactacacaatggattgggtgcgacaggcccccggaaagggactggagtgggtgggcgatgtcaaccctaattctggcgggagtatctacaaccagcggttcaaggggagattcactttttcagtggacagaagcaaaaacaccctgtatctgcagatgaacagcctgagggccgaagataccgctgtctactattgcgctcgcaatctgggccccagtttctactttgactattgggggcagggaaccctggtgacagtcagctccgctagcactaaggggccttccgtgtttccactggctccctctagtaaatccacctctggaggcacagctgcactgggatgtctggtgaaggattacttccctgaaccagtcacagtgagttggaactcaggggctctgacaagtggagtccatacttttcccgcagtgctgcagtcaagcggactgtactccctgtcctctgtggtcaccgtgcctagttcaagcctgggcacccagacatatatctgcaacgtgaatcacaagccatcaaatacaaaagtcgacaagaaagtggagcccaagagctgtgataaaactcatacctgcccaccttgtccggcgccagaactgctgggaggaccaagcgtgttcctgtttccacccaagcctaaagacaccctgatgatttcccggactcctgaggtcacctgcgtggtcgtggacgtgtctcacgaggaccccgaagtcaagttcaactggtacgtggatggcgtcgaagtgcataatgccaagaccaaaccccgggaggaacagtacaactctacctatagagtcgtgagtgtcctgacagtgctgcaccaggactggctgaatgggaaggagtataagtgtaaagtgagcaacaaagccctgcccgccccaatcgaaaaaacaatctctaaagcaaaaggacagcctcgcgaaccacaggtctacgtctaccccccatcaagagatgaactgacaaaaaatcaggtctctctgacatgcctggtcaaaggattctacccttccgacatcgccgtggagtgggaaagtaacggccagcccgagaacaattacaagaccacaccccctgtcctggactctgatgggagtttcgctctggtgtcaaagctgaccgtcgataaaagccggtggcagcagggcaatgtgtttagctgctccgtcatgcacgaagccctgcacaatcactacacacagaagtccctgagcctgagccctggc

SEQ ID NO: 38 - protein, 119 aa, synthetic construct
  REGION 1..119: note = Artificial sequence
EVQLVESGGGLVQPGGSLRLSCAASGFTFADYTMDWVRQAPGKGLEWVGDVNPNSGGSIYNQRFKGRFTFSVDRSKNTLYLQMNSLRAEDTAVYYCARNLGPSFYFDYWGQGTLVTVSS

SEQ ID NO: 39 - protein, 8 aa, synthetic construct
  REGION 1..8: note = Artificial sequence
GFTFADYT

SEQ ID NO: 40 - protein, 12 aa, synthetic construct
  REGION 1..12: note = Artificial sequence
ARNLGPSFYFDY

SEQ ID NO: 41 - protein, 8 aa, synthetic construct
  REGION 1..8: note = Artificial sequence
VNPNSGGS

SEQ ID NO: 42 - protein, 226 aa, synthetic construct
  REGION 1..226: note = Artifcial sequence
YPYDVPDYATGSDIQMTQSPSSLSASVGDRVTITCKASQDVSIGVAWYQQKPGKAPKLLIYSASYRYTGVPSRFSGSGSGTDFTLTISSLQPEDFATYYCQQYYIYPYTFGQGTKVEIKRTVAAPSVFIFPPSDEELKSGTASVVCLLNNFYPREAKVQWKVDNALQSGNSEESVTEQDSKDSTYSLSSTLELSKADYEKHKVYACEVTHQGLSSPVTKSFNRGEC

SEQ ID NO: 43 - DNA, 678 bp, synthetic construct
  misc_feature 1..678: note = Artificial sequence
  source 1..678: mol_type = other DNA
tatccctacgatgtgcctgactacgctactggctccgatatccagatgacccagtctccaagctccctgagtgcatcagtgggggaccgagtcaccatcacatgcaaggcttcccaggatgtgtctattggagtcgcatggtaccagcagaagccaggcaaagcacccaagctgctgatctacagcgcctcctaccggtatactggggtgccttccagattctctggcagtgggtcaggaaccgactttactctgaccatctctagtctgcagcccgaggatttcgccacctactattgccagcagtactatatctacccttatacctttggccaggggacaaaagtggagatcaagaggacagtggccgctccaagtgtcttcatttttcccccttccgacgaagagctgaaaagtggaactgcttcagtggtctgtctgctgaacaatttctacccccgcgaagccaaagtgcagtggaaggtcgataacgctctgcagagcggcaattccgaggagtctgtgacagaacaggacagtaaagattcaacttatagcctgtcaagcacactggagctgtctaaggcagactacgagaagcacaaagtgtatgcctgcgaagtcacccatcaggggctgtcctctcccgtgacaaagagctttaacagaggagagtgt

SEQ ID NO: 44 - protein, 107 aa, synthetic construct [sequence omitted]

SEQ ID NO: 45 - protein, 481 aa, synthetic construct
  REGION 1..481: note = Artificial sequence
DIQMTQSPSSLSASVGDRVTITCRASQDVNTAVAWYQQKPGKAPKLLIYSASFLYSGVPSRFSGSRSGTDFTLTISSLQPEDFATYYCQQHYTTPPTFGQGTKVEIKGGSGGGSGGGSGGGSGGGSGEVQLVESGGGLVQPGGSLRLSCAASGFNIKDTYIHWVRQAPGKGLEWVARIYPTNGYTRYADSVKGRFTISADTSKNTAYLQMNSLRAEDTAVYYCSRWGGDGFYAMDYWGQGTLVTVSSAAEPKSSDKTHTCPPCPAPELLGGPSVFLFPPKPKDTLMISRTPEVTCVVVDVSHEDPEVKFNWYVDGVEVHNAKTKPREEQYNSTYRVVSVLTVLHQDWLNGKEYKCKVSNKALPAPIEKTISKAKGQPREPQVYTYPPSRDELTKNQVSLTCLVKGFYPSDIAVEWESNGQPENNYKTTPPVLDEDGSFALVSKLTVDKSRWQQGNVFSCSVMHEALHNHYTQKSLSLSPGK

SEQ ID NO: 46 - DNA, 1443 bp, synthetic construct
  misc_feature 1..1443: note = Artificial sequence
  source 1..1443: mol_type = other DNA
gacatccagatgacccagtctccatcctccctgtctgcatctgtaggagacagagtcaccatcacttgccgggcaagtcaggacgttaacaccgctgtagcttggtatcagcagaaaccagggaaagcccctaagctcctgatctattctgcatcctttttgtacagtggggtcccatcaaggttcagtggcagtcgatctgggacagatttcactctcaccatcagcagtctgcaacctgaagattttgcaacttactactgtcaacagcattacactaccccacccactttcggccaagggaccaaagtggagatcaaaggtggttctggtggtggttctggtggtggttctggtggtggttctggtggtggttctggtgaagtgcagctggtggagtctgggggaggcttggtacagcctggcgggtccctgagactctcctgtgcagcctctggattcaacattaaagatacttatatccactgggtccggcaagctccagggaagggcctggagtgggtcgcacgtatttatcccacaaatggttacacacggtatgcggactctgtgaagggccgattcaccatctccgcagacacttccaagaacaccgcgtatctgcaaatgaacagtctgagagctgaggacacggccgtttattactgttcaagatggggcggagacggtttctacgctatggactactggggccaagggaccctggtcaccgtctcctcagccgccgagcccaagagcagcgataagacccacacctgccctccctgtccagctccagaactgctgggaggacctagcgtgttcctgtttccccctaagccaaaagacactctgatgatttccaggactcccgaggtgacctgcgtggtggtggacgtgtctcacgaggaccccgaagtgaagttcaactggtacgtggatggcgtggaagtgcataatgctaagacaaaaccaagagaggaacagtacaactccacttatcgcgtcgtgagcgtgctgaccgtgctgcaccaggactggctgaacgggaaggagtataagtgcaaagtcagtaataaggccctgcctgctccaatcgaaaaaaccatctctaaggccaaaggccagccaagggagccccaggtgtacacatacccacccagcagagacgaactgaccaagaaccaggtgtccctgacatgtctggtgaaaggcttctatcctagtgatattgctgtggagtgggaatcaaatggacagccagagaacaattacaagaccacacctccagtgctggacgaggatggcagcttcgccctggtgtccaagctgacagtggataaatctcgatggcagcaggggaacgtgtttagttgttcagtgatgcatgaagccctgcacaatcattacactcagaagagcctgtccctgtctcccggcaaa

SEQ ID NO: 47 - protein, 107 aa, synthetic construct [sequence omitted]

SEQ ID NO: 48 - protein, 120 aa, synthetic construct [sequence omitted]

SEQ ID NO: 49 - protein, 481 aa, synthetic construct
  REGION 1..481: note = Artificial sequence
DIQMTQSPSSLSASVGDRVTITCRASQDVNTAVAWYQQKPGKAPKLLIYSASFLYSGVPSRFSGSRSGTDFTLTISSLQPEDFATYYCQQHYTTPPTFGQGTKVEIKGGSGGGSGGGSGGGSGGGSGEVQLVESGGGLVQPGGSLRLSCAASGFNIKDTYIHWVRQAPGKGLEWVARIYPTNGYTRYADSVKGRFTISADTSKNTAYLQMNSLRAEDTAVYYCSRWGGDGFYAMDYWGQGTLVTVSSAAEPKSSDKTHTCPPCPAPELLGGPSVFLFPPKPKDTLMISRTPEVTCVVVDVSHEDPEVKFNWYVDGVEVHNAKTKPREEQYNSTYRVVSVLTVLHQDWLNGKEYKCKVSNKALPAPIEKTISKAKGQPREPQVYTLPPSRDELTKNQVSLICLVKGFYPSDIAVEWESNGQPENRYMTWPPVLDSDGSFFLYSKLTVDKSRWQQGNVFSCSVMHEALHNHYTQKSLSLSPGK

SEQ ID NO: 50 - DNA, 1443 bp, synthetic construct
  misc_feature 1..1443: note = Artificial sequence
  source 1..1443: mol_type = other DNA
gacatccagatgacccagtctccatcctccctgtctgcatctgtaggagacagagtcaccatcacttgccgggcaagtcaggacgttaacaccgctgtagcttggtatcagcagaaaccagggaaagcccctaagctcctgatctattctgcatcctttttgtacagtggggtcccatcaaggttcagtggcagtcgatctgggacagatttcactctcaccatcagcagtctgcaacctgaagattttgcaacttactactgtcaacagcattacactaccccacccactttcggccaagggaccaaagtggagatcaaaggtggttctggtggtggttctggtggtggttctggtggtggttctggtggtggttctggtgaagtgcagctggtggagtctgggggaggcttggtacagcctggcgggtccctgagactctcctgtgcagcctctggattcaacattaaagatacttatatccactgggtccggcaagctccagggaagggcctggagtgggtcgcacgtatttatcccacaaatggttacacacggtatgcggactctgtgaagggccgattcaccatctccgcagacacttccaagaacaccgcgtatctgcaaatgaacagtctgagagctgaggacacggccgtttattactgttcaagatggggcggagacggtttctacgctatggactactggggccaagggaccctggtcaccgtctcctcagccgccgagcccaagagcagcgataagacccacacctgccctccctgtccagctccagaactgctgggaggacctagcgtgttcctgtttccccctaagccaaaagacactctgatgatttccaggactcccgaggtgacctgcgtggtggtggacgtgtctcacgaggaccccgaagtgaagttcaactggtacgtggatggcgtggaagtgcataatgctaagacaaaaccaagagaggaacagtacaactccacttatcgcgtcgtgagcgtgctgaccgtgctgcaccaggactggctgaacgggaaggagtataagtgcaaagtcagtaataaggccctgcctgctccaatcgaaaaaaccatctctaaggccaaaggccagccaagggagccccaggtgtacacactgccacccagcagagacgaactgaccaagaaccaggtgtccctgatctgtctggtgaaaggcttctatcctagtgatattgctgtggagtgggaatcaaatggacagccagagaacagatacatgacctggcctccagtgctggacagcgatggcagcttcttcctgtattccaagctgacagtggataaatctcgatggcagcaggggaacgtgtttagttgttcagtgatgcatgaagccctgcacaatcattacactcagaagagcctgtccctgtctcccggcaaa

SEQ ID NO: 51 - protein, 107 aa, synthetic construct [sequence omitted]

SEQ ID NO: 52 - protein, 120 aa, synthetic construct [sequence omitted]

SEQ ID NO: 53 - protein, 448 aa, synthetic construct
  REGION 1..448: note = Artificial sequence
EVQLVESGGGLVQPGGSLRLSCAASGFTFTDYTMDWVRQAPGKGLEWVADVNPNSGGSIYNQRFKGRFTLSVDRSKNTLYLQMNSLRAEDTAVYYCARNLGPSFYFDYWGQGTLVTVSSASTKGPSVFPLAPSSKSTSGGTAALGCLVKDYFPEPVTVSWNSGALTSGVHTFPAVLQSSGLYSLSSVVTVPSSSLGTQTYICNVNHKPSNTKVDKKVEPKSCDKTHTCPPCPAPELLGGPSVFLFPPKPKDTLMISRTPEVTCVVVDVSHEDPEVKFNWYVDGVEVHNAKTKPREEQYNSTYRVVSVLTVLHQDWLNGKEYKCKVSNKALPAPIEKTISKAKGQPREPQVYVLPPSRDELTKNQVSLLCLVKGFYPSDIAVEWESNGQPENNYLTWPPVLDSDGSFFLYSKLTVDKSRWQQGNVFSCSVMHEALHNHYTQKSLSLSPG

SEQ ID NO: 54 - DNA, 1344 bp, synthetic construct
  misc_feature 1..1344: note = Artificial sequence
  source 1..1344: mol_type = other DNA
gaagtgcagctggtcgaatctggaggaggactggtgcagccaggagggtccctgcgcctgtcttgcgccgctagtggcttcacttttaccgactacaccatggattgggtgcgacaggcacctggaaagggcctggagtgggtcgccgatgtgaacccaaatagcggaggctccatctacaaccagcggttcaagggccggttcaccctgtcagtggaccggagcaaaaacaccctgtatctgcagatgaatagcctgcgagccgaagatactgctgtgtactattgcgcccggaatctggggccctccttctactttgactattgggggcagggaactctggtcaccgtgagctccgcctccaccaagggaccttctgtgttcccactggctccctctagtaaatccacatctgggggaactgcagccctgggctgtctggtgaaggactacttcccagagcccgtcacagtgtcttggaacagtggcgctctgacttctggggtccacacctttcctgcagtgctgcagtcaagcgggctgtacagcctgtcctctgtggtcaccgtgccaagttcaagcctgggaacacagacttatatctgcaacgtgaatcacaagccatccaatacaaaagtcgacaagaaagtggaacccaagtcttgtgataaaacccatacatgccccccttgtcctgcaccagagctgctgggaggaccaagcgtgttcctgtttccacccaagcctaaagatacactgatgattagtaggaccccagaagtcacatgcgtggtcgtggacgtgagccacgaggaccccgaagtcaagtttaactggtacgtggacggcgtcgaggtgcataatgccaagactaaacccagggaggaacagtacaacagtacctatcgcgtcgtgtcagtcctgacagtgctgcatcaggattggctgaacgggaaagagtataagtgcaaagtgagcaataaggctctgcccgcacctatcgagaaaacaatttccaaggcaaaaggacagcctagagaaccacaggtgtacgtgctgcctccatcaagggatgagctgacaaagaaccaggtcagcctgctgtgtctggtgaaaggattctatccctctgacattgctgtggagtgggaaagtaatggccagcctgagaacaattacctgacctggccccctgtgctggactcagatggcagcttctttctgtatagcaagctgaccgtcgacaaatcccggtggcagcaggggaatgtgtttagttgttcagtcatgcacgaggcactgcacaaccattacacccagaagtcactgtcactgtcaccaggg

SEQ ID NO: 55 - protein, 119 aa, synthetic construct [sequence omitted]

SEQ ID NO: 56 - protein, 448 aa, synthetic construct
  REGION 1..448: note = Artificial sequence
EVQLVESGGGLVQPGGSLRLSCAASGFTFTDYTMDWVRQAPGKGLEWVADVNPNSGGSIYNQRFKGRFTLSVDRSKNTLYLQMNSLRAEDTAVYYCARNLGPSFYFDYWGQGTLVTVSSASTKGPSVFPLAPSSKSTSGGTAALGCLVKDYFPEPVTVSWNSGALTSGVHTFPAVLQSSGLYSLSSVVTVPSSSLGTQTYICNVNHKPSNTKVDKKVEPKSCDKTHTCPPCPAPELLGGPSVFLFPPKPKDTLMISRTPEVTCVVVDVSHEDPEVKFNWYVDGVEVHNAKTKPREEQYNSTYRVVSVLTVLHQDWLNGKEYKCKVSNKALPAPIEKTISKAKGQPREPQVYVYPPSRDELTKNQVSLTCLVKGFYPSDIAVEWESNGQPENNYKTTPPVLDSDGSFALVSKLTVDKSRWQQGNVFSCSVMHEALHNHYTQKSLSLSPG

SEQ ID NO: 57 - DNA, 1344 bp, synthetic construct
  misc_feature 1..1344: note = Artificial sequence
  source 1..1344: mol_type = other DNA
gaagtgcagctggtcgaatctggaggaggactggtgcagccaggagggtccctgcgcctgtcttgcgccgctagtggcttcacttttaccgactacaccatggattgggtgcgacaggcacctggaaagggcctggagtgggtcgccgatgtgaacccaaatagcggaggctccatctacaaccagcggttcaagggccggttcaccctgtcagtggaccggagcaaaaacaccctgtatctgcagatgaatagcctgcgagccgaagatactgctgtgtactattgcgcccggaatctggggccctccttctactttgactattgggggcagggaactctggtcaccgtgagctccgcctccaccaagggaccttctgtgttcccactggctccctctagtaaatccacatctgggggaactgcagccctgggctgtctggtgaaggactacttcccagagcccgtcacagtgtcttggaacagtggcgctctgacttctggggtccacacctttcctgcagtgctgcagtcaagcgggctgtacagcctgtcctctgtggtcaccgtgccaagttcaagcctgggaacacagacttatatctgcaacgtgaatcacaagccatccaatacaaaagtcgacaagaaagtggaacccaagtcttgtgataaaacccatacatgccccccttgtcctgcaccagagctgctgggaggaccaagcgtgttcctgtttccacccaagcctaaagatacactgatgattagtaggaccccagaagtcacatgcgtggtcgtggacgtgagccacgaggaccccgaagtcaagtttaactggtacgtggacggcgtcgaggtgcataatgccaagactaaacccagggaggaacagtacaacagtacctatcgcgtcgtgtcagtcctgacagtgctgcatcaggattggctgaacgggaaagagtataagtgcaaagtgagcaataaggctctgcccgcacctatcgagaaaacaatttccaaggcaaaaggacagcctagagaaccacaggtgtacgtgtatcctccatcaagggatgagctgacaaagaaccaggtcagcctgacttgtctggtgaaaggattctatccctctgacattgctgtggagtgggaaagtaatggccagcctgagaacaattacaagaccacaccccctgtgctggactcagatggcagcttcgcgctggtgagcaagctgaccgtcgacaaatcccggtggcagcaggggaatgtgtttagttgttcagtcatgcacgaggcactgcacaaccattacacccagaagtcactgtcactgtcaccaggg

SEQ ID NO: 58 - protein, 119 aa, synthetic construct [sequence omitted]

SEQ ID NO: 59 - protein, 475 aa, synthetic construct
  REGION 1..475: note = Artificial sequence
DIQMTQSPSSLSASVGDRVTITCKASQDVSIGVAWYQQKPGKAPKLLIYSASYRYTGVPSRFSGSGSGTDFTLTISSLQPEDFATYYCQQYYIYPYTFGQGTKVEIKGGGGSGGGGSGGGGSEVQLVESGGGLVQPGGSLRLSCAASGFTFTDYTMDWVRQAPGKGLEWVADVNPNSGGSIYNQRFKGRFTLSVDRSKNTLYLQMNSLRAEDTAVYYCARNLGPSFYFDYWGQGTLVTVSSAAEPKSSDKTHTCPPCPAPELLGGPSVFLFPPKPKDTLMISRTPEVTCVVVDVSHEDPEVKFNWYVDGVEVHNAKTKPREEQYNSTYRVVSVLTVLHQDWLNGKEYKCKVSNKALPAPIEKTISKAKGQPREPQVYVYPPSRDELTKNQVSLTCLVKGFYPSDIAVEWESNGQPENNYKTTPPVLDSDGSFALVSKLTVDKSRWQQGNVFSCSVMHEALHNHYTQKSLSLSPGK

SEQ ID NO: 60 - DNA, 1425 bp, synthetic construct
  misc_feature 1..1425: note = Artificial sequence
  source 1..1425: mol_type = other DNA
gacattcagatgacccagagccctagctccctgagtgcctcagtcggggacagggtgactatcacctgcaaggcttcacaggatgtcagcattggcgtggcatggtaccagcagaagccagggaaagcacccaagctgctgatctatagcgcctcctacaggtatacaggcgtgccatcccgcttctctggcagtgggtcaggaactgactttacactgactatttctagtctgcagcccgaagatttcgccacatactattgccagcagtactatatctacccttatacttttggccaggggaccaaagtggagattaagggcggaggaggctccggaggaggagggtctggaggaggaggaagtgaggtccagctggtggaatctggaggaggactggtgcagccaggagggtccctgaggctgtcttgtgccgctagtggcttcacctttacagactacacaatggattgggtgcgccaggcaccaggaaagggactggaatgggtcgctgatgtgaaccctaatagcggaggctccatctacaaccagcggttcaaaggacggttcaccctgtcagtggaccggagcaagaacaccctgtatctgcagatgaacagcctgagagccgaggatactgctgtgtactattgcgccaggaatctgggcccaagcttctactttgactattgggggcagggaacactggtcactgtgtcaagcgcagccgaacccaaatcctctgataagactcacacctgcccaccttgtccagctccagagctgctgggaggacctagcgtgttcctgtttccacccaagccaaaagacactctgatgatttctagaacccctgaagtgacatgtgtggtcgtggacgtcagtcacgaggaccccgaagtcaaattcaactggtacgtggatggcgtcgaggtgcataatgccaagaccaaaccccgagaggaacagtacaactcaacctatcgggtcgtgagcgtcctgacagtgctgcatcaggactggctgaacggcaaggagtataagtgcaaagtgagcaacaaggctctgcctgcaccaatcgagaagaccatttccaaggctaaagggcagccccgcgaacctcaggtctacgtgtatcctccaagccgagatgagctgacaaaaaaccaggtctccctgacttgtctggtgaagggattttacccaagtgacatcgcagtggagtgggaatcaaatggccagcccgaaaacaattataagaccacaccccctgtgctggactctgatgggagtttcgcactggtctccaaactgaccgtggacaagtctcggtggcagcagggaaacgtctttagctgttccgtgatgcacgaggccctgcacaatcattacacacagaaatctctgagtctgtcacctggcaag

SEQ ID NO: 61 - protein, 107 aa, synthetic construct [sequence omitted]

SEQ ID NO: 62 - protein, 119 aa, synthetic construct [sequence omitted]

SEQ ID NO: 63 - protein, 480 aa, synthetic construct
  REGION 1..480: note = Artificial sequence
DIQMTQSPSSLSASVGDRVTITCRASQDVNTAVAWYQQKPGKAPKLLIYSASFLYSGVPSRFSGSRSGTDFTLTISSLQPEDFATYYCQQHYTTPPTFGQGTKVEIKGGSGGGSGGGSGGGSGGGSGEVQLVESGGGLVQPGGSLRLSCAASGFNIKDTYIHWVRQAPGKGLEWVARIYPTNGYTRYADSVKGRFTISADTSKNTAYLQMNSLRAEDTAVYYCSRWGGDGFYAMDYWGQGTLVTVSSAAEPKSSDKTHTCPPCPAPELLGGPSVFLFPPKPKDTLMISRTPEVTCVVVDVSHEDPEVKFNWYVDGVEVHNAKTKPREEQYNSTYRVVSVLTVLHQDWLNGKEYKCKVSNKALPAPIEKTISKAKGQPREPQVYVLPPSRDELTKNQVSLLCLVKGFYPSDIAVEWESNGQPENNYLTWPPVLDSDGSFFLYSKLTVDKSRWQQGNVFSCSVMHEALHNHYTQKSLSLSPG

SEQ ID NO: 64 - DNA, 1440 bp, synthetic construct
  misc_feature 1..1440: note = Artificial sequence
  source 1..1440: mol_type = other DNA
gacattcagatgacacagagccccagctccctgagtgcttcagtcggcgacagggtgactatcacctgccgcgcatcccaggatgtcaacaccgctgtggcatggtaccagcagaagcctggaaaagccccaaagctgctgatctacagcgcttccttcctgtattctggcgtgccaagtcggttttctggaagtagatcaggcactgacttcacactgactatctctagtctgcagcccgaagattttgccacctactattgccagcagcactataccacaccccctacattcggacagggcactaaagtggagattaagggcgggtcaggcggagggagcggaggagggtccggaggagggtctggaggagggagtggagaggtccagctggtggaatctggaggaggactggtgcagcctggaggctcactgcgactgagctgtgccgcttccggctttaacatcaaagacacatacattcattgggtcaggcaggcaccagggaagggactggaatgggtggcccgcatctatcccacaaatgggtacactcgatatgccgacagcgtgaaaggacggtttaccatttctgctgataccagtaagaacacagcatacctgcagatgaacagcctgcgcgcagaggatacagccgtgtactattgcagtcgatgggggggagacggcttctacgccatggattattggggccaggggactctggtcaccgtgtcaagcgcagccgaacctaaatcctctgacaagacccacacatgcccaccctgtcctgctccagagctgctgggaggaccatccgtgttcctgtttcctccaaagcctaaagatacactgatgattagccgcactcccgaagtcacctgtgtggtcgtggacgtgtcccacgaggaccccgaagtcaagttcaactggtacgtggacggcgtcgaggtgcataatgccaagactaaaccaagagaggaacagtacaattcaacctatagggtcgtgagcgtcctgacagtgctgcatcaggattggctgaacggcaaggagtataagtgcaaagtgtctaacaaggccctgcccgctcctatcgagaagactattagcaaggcaaaagggcagccacgggaaccccaggtctacgtgctgccccctagcagagacgagctgaccaaaaaccaggtctccctgctgtgtctggtgaagggcttttatcctagtgatatcgctgtggagtgggaatcaaatgggcagccagaaaacaattacctgacatggccacccgtgctggacagcgatgggtccttctttctgtattccaaactgactgtggacaagtctagatggcagcagggaaacgtcttcagctgttccgtgatgcacgaggccctgcacaatcattacacccagaagtctctgagtctgtcacccggc

SEQ ID NO: 65 - protein, 107 aa, synthetic construct [sequence omitted]

SEQ ID NO: 66 - protein, 120 aa, synthetic construct [sequence omitted]

SEQ ID NO: 67 - protein, 6 aa, synthetic construct
  REGION 1..6: note = Artificial sequence
QDVNTA

SEQ ID NO: 68 - skipped

SEQ ID NO: 69 - protein, 9 aa, synthetic construct
  REGION 1..9: note = Artificial sequence
QQHYTTPPT

SEQ ID NO: 70 - protein, 8 aa, synthetic construct
  REGION 1..8: note = Artificial sequence
GFNIKDTY

SEQ ID NO: 71 - protein, 8 aa, synthetic construct
  REGION 1..8: note = Artificial sequence
IYPTNGYT

SEQ ID NO: 72 - protein, 13 aa, synthetic construct
  REGION 1..13: note = Artificial sequence
SRWGGDGFYAMDY

SEQ ID NO: 73 - protein, 8 aa, synthetic construct
  REGION 1..8: note = Artificial sequence
VNPNSGYS

SEQ ID NO: 74 - protein, 8 aa, synthetic construct
  REGION 1..8: note = Artificial sequence
GFTFQDYT

SEQ ID NO: 75 - protein, 12 aa, synthetic construct
  REGION 1..12: note = Artificial sequence
ARNLGPWFYFDY

SEQ ID NO: 76 - protein, 9 aa, synthetic construct
  REGION 1..9: note = Artificial sequence
QQYYIYPGT

SEQ ID NO: 77 - protein, 8 aa, synthetic construct
  REGION 1..8: note = Artificial sequence
GFTFYDYT

SEQ ID NO: 78 - protein, 119 aa, synthetic construct
  REGION 1..119: note = Artificial sequence
EVQLVESGGGLVQPGGSLRLSCAASGFTFADYTMDWVRQAPGKGLEWVADVNPNSGGSIYNQRFKGRFTLSVDRSKNTLYLQMNSLRAEDTAVYYCARNLGPSFYFDYWGQGTLVTVSS

SEQ ID NO: 79 - protein, 107 aa, synthetic construct; identical to SEQ ID NO: 26
  REGION 1..107: note = Artificial sequence

SEQ ID NO: 80 - protein, 119 aa, synthetic construct
  REGION 1..119: note = Artificial sequence
EVQLVESGGGLVQPGGSLRLSCAASGFTFTDYTMDWVRQAPGKGLEWVADVNPNSGYSIYNQRFKGRFTLSVDRSWNTLYLQMNSLRAEDTAVYYCARNLGPSFYFDYWGQGTLVTVSS

SEQ ID NO: 81 - protein, 107 aa, synthetic construct [sequence omitted]

SEQ ID NO: 82 - protein, 119 aa, synthetic construct
  REGION 1..119: note = Artificial sequence
EVQLVESGGGLVQPGGSLRLSCAASGFTFQDYTMDWVRQAPGKGLEWVADVNPNSGGSIYNQRFKGRFTLSVDRSKNTLYLQMNSLRAEDTAVYYCARNLGPWFYFDYWGQGTLVTVSS

SEQ ID NO: 83 - protein, 119 aa, synthetic construct
  REGION 1..119: note = Artificial sequence
EVQLVESGGGLVQPGGSLRLSCAASGFTFQDYTMDWVRQAPGKGLEWVADVNPNSGGSIYNQRFKGRFTLSVDRSKNTLYLQMNSLRAEDTAVYYCARNLGPSFYFDYWGQGTLVTVSS

SEQ ID NO: 84 - protein, 107 aa, synthetic construct
  REGION 1..107: note = Artificial sequence
DIQMTQSPSSLSASVGDRVTITCKASQDVSIGVAWYQQKPGKAPKLLIWSASYRYTGVPSRFSGSGSGTDFTLTISSLQPEDFATYYCQQYYIYPGTFGQGTKVEIK

SEQ ID NO: 85 - protein, 119 aa, synthetic construct
  REGION 1..119: note = Artificial sequence
EVQLVESGGGLVQPGGSLRLSCAASGFTFQDYTMDWVRQAPGKGLEWVADVNPNSGGSIYNQRFKGRFTLSVDRSWNTLYLQMNSLRAEDTAVYYCARNLGPSFYFDYWGQGTLVTVSS

SEQ ID NO: 86 - protein, 119 aa, synthetic construct
  REGION 1..119: note = Artificial sequence
EVQLVESGGGLVQPGGSLRLSCAASGFTFYDYTMDWVRQAPGKGLEWVADVNPNSGGSIYNQRFKGRFTLSVDRSWNTLYLQMNSLRAEDTAVYYCARNLGPSFYFDYWGQGTLVTVSS

SEQ ID NO: 87 - protein, 119 aa, synthetic construct
  REGION 1..119: note = Artificial sequence
EVQLVESGGGLVQPGGSLRLSCAASGFTFQDYTMDWVRQAPGKGLEWVADVNPNSGYSIYNQRFKGRFTLSVDRSKNTLYLQMNSLRAEDTAVYYCARNLGPWFYFDYWGQGTLVTVSS

SEQ ID NO: 88 - protein, 107 aa, synthetic construct
  REGION 1..107: note = Artificial sequence
DIQMTQSPSSLSASVGDRVTITCKASQDVSIGVAWYQQKPGKAPKLLIWSASYRYTGVPSRFSGSGSGTDFTLTISSLQPEDFATYYCQQYYIYPYTFGQGTKVEIK

SEQ ID NO: 89 - protein, 119 aa, synthetic construct
  REGION 1..119: note = Artificial sequence
EVQLVESGGGLVQPGGSLRLSCAASGFTFQDYTMDWVRQAPGKGLEWVADVNPNSGYSIYNQRFKGRFTLSVDRSKNTLYLQMNSLRAEDTAVYYCARNLGPSFYFDYWGQGTLVTVSS